European Patent Application EP 4 241 789 A2, published September 13, 2023. Title: PROTEIN-DRUG CONJUGATE AND SITE-SPECIFIC CONJUGATING METHOD. Applicant: Harbour Biomed (Shanghai) Co., Ltd. Application 21731365.9. The sequence listing filed with the application follows.

SEQUENCE LISTING (149 sequences)

SEQ ID NO: 1 - protein, 25 aa, Artificial Sequence
  PR000020 HFWR1 Chothia, PR001046 HFWR1 Chothia, PR004433 HFWR1 Chothia
EVQLVETGGGLIQPGGSLRLSCAAS

SEQ ID NO: 2 - protein, 25 aa, Artificial Sequence
  PR000184 HFWR1 Chothia
EVQLVESGGGLIQPGGSLRLSCAVS

SEQ ID NO: 3 - protein, 25 aa, Artificial Sequence
  PR000453 HFWR1 Chothia
EVQLVESGGGLVQAGGSLRLSCAAS

SEQ ID NO: 4 - protein, 25 aa, Artificial Sequence
  PR000759 HFWR1 Chothia
EVQLVESGGGVVQPGRSLRLSCAAS

SEQ ID NO: 5 - protein, 25 aa, Artificial Sequence
  PR002129 HFWR1 Chothia
QVQLVQSGGGVVQPGRSLRLSCAAS

SEQ ID NO: 6 - protein, 25 aa, Artificial Sequence
  PR004432 HFWR1 Chothia
EVQLQQSGPGLVKPSQTLSLTCAIS

SEQ ID NO: 7 - protein, 7 aa, Artificial Sequence
  PR000020 HCDR1 Chothia
GLNVSRH

SEQ ID NO: 8 - protein, 7 aa, Artificial Sequence
  PR000184 HCDR1 Chothia
GFTVSKN

SEQ ID NO: 9 - protein, 4 aa, Artificial Sequence
  PR000453 HCDR1 Chothia
GRTF

SEQ ID NO: 10 - protein, 7 aa, Artificial Sequence
  PR000759 HCDR1 Chothia
GFTFSSF

SEQ ID NO: 11 - protein, 7 aa, Artificial Sequence
  PR001046 HCDR1 Chothia
GFTVSDN

SEQ ID NO: 12 - protein, 7 aa, Artificial Sequence
  PR002129 HCDR1 Chothia
GFTFSSY

SEQ ID NO: 13 - protein, 9 aa, Artificial Sequence
  PR004432 HCDR1 Chothia
GDSVSNNYA

SEQ ID NO: 14 - protein, 7 aa, Artificial Sequence
  PR004433 HCDR1 Chothia
GFTVSDS

SEQ ID NO: 15 - protein, 19 aa, Artificial Sequence
  PR000020 HFWR2 Chothia
YLSWVRQAPGKGLEWVAVI

SEQ ID NO: 16 - protein, 19 aa, Artificial Sequence
  PR000184 HFWR2 Chothia
YMSWVRQAPGKGLEWVSVV

SEQ ID NO: 17 - protein, 19 aa, Artificial Sequence
  PR000453 HFWR2 Chothia
TMGWFRQAPGKEREFVAAI

SEQ ID NO: 18 - protein, 19 aa, Artificial Sequence
  PR000759 HFWR2 Chothia
AFHWVRQAPGKGLEGVAVI

SEQ ID NO: 19 - protein, 19 aa, Artificial Sequence
  PR001046 HFWR2 Chothia, PR004433 HFWR2 Chothia
YMTWVRQAPGKGLEWVSVI

SEQ ID NO: 20 - protein, 19 aa, Artificial Sequence
  PR002129 HFWR2 Chothia
GMHWVRQAPGKGLEWVAVI

SEQ ID NO: 21 - protein, 19 aa, Artificial Sequence
  PR004432 HFWR2 Chothia
AWNWIRQSPSRGLEWLGRT

SEQ ID NO: 22 - protein, 5 aa, Artificial Sequence
  PR000020 HCDR2 Chothia
YSGGG

SEQ ID NO: 23 - protein, 5 aa, Artificial Sequence
  PR000184 HCDR2 Chothia
YSGGS

SEQ ID NO: 24 - protein, 6 aa, Artificial Sequence
  PR000453 HCDR2 Chothia
SLSPTL

SEQ ID NO: 25 - protein, 6 aa, Artificial Sequence
  PR000759 HCDR2 Chothia
WYDGRN

SEQ ID NO: 26 - protein, 5 aa, Artificial Sequence
  PR001046 HCDR2 Chothia
FSGGN

SEQ ID NO: 27 - protein, 6 aa, Artificial Sequence
  PR002129 HCDR2 Chothia
WYDGSN

SEQ ID NO: 28 - protein, 7 aa, Artificial Sequence
  PR004432 HCDR2 Chothia
YYRSKWY

SEQ ID NO: 29 - protein, 5 aa, Artificial Sequence
  PR004433 HCDR2 Chothia
FSGGR

SEQ ID NO: 30 - protein, 41 aa, Artificial Sequence
  PR000020 HFWR3 Chothia
IEYVDSVKGRFTISRDNANNTLYLQMRSLRTEDSAVYYCAR

SEQ ID NO: 31 - protein, 41 aa, Artificial Sequence
  PR000184 HFWR3 Chothia
KTYADSVKGRFTISRDNSKNTLYLQMNSLRAEDTAVYYCAR

SEQ ID NO: 32 - protein, 41 aa, Artificial Sequence
  PR000453 HFWR3 Chothia
AYYAESVKGRFTISRDNAKNTVVLQMNSLKPEDTALYYCAA

SEQ ID NO: 33 - protein, 41 aa, Artificial Sequence
  PR000759 HFWR3 Chothia
ENYADSVKGRFTISRDNSKNMLYLQMNSLRAEDTAVYYCAR

SEQ ID NO: 34 - protein, 41 aa, Artificial Sequence
  PR001046 HFWR3 Chothia
TYYADSVKGRFTISRDNAKNTLYLQMNSLRAEDTALYYCAR

SEQ ID NO: 35 - protein, 41 aa, Artificial Sequence
  PR002129 HFWR3 Chothia
KDYADSVKGRFTISRDTSKNTLYLQMNSLRAEDTAVYYCAR

SEQ ID NO: 36 - protein, 41 aa, Artificial Sequence
  PR004432 HFWR3 Chothia
NDYAVSVKSRITINPDTSKNQFSLQLNRVTPEDTAVYYCAR

SEQ ID NO: 37 - protein, 41 aa, Artificial Sequence
  PR004433 HFWR3 Chothia
TYYSDSVKGRFTISRDNAKNTLYLQMNSLRAEDTALYYCAR

SEQ ID NO: 38 - protein, 10 aa, Artificial Sequence
  PR000020 HCDR3 Chothia
AIPRPHGSDI

SEQ ID NO: 39 - protein, 11 aa, Artificial Sequence
  PR000184 HCDR3 Chothia
AVPHSPSSFDI

SEQ ID NO: 40 - protein, 12 aa, Artificial Sequence
  PR000453 HCDR3 Chothia
DRKSVMSIRPDY

SEQ ID NO: 41 - protein, 13 aa, Artificial Sequence
  PR000759 HCDR3 Chothia
GRGVLGDTRAFDI

SEQ ID NO: 42 - protein, 14 aa, Artificial Sequence
  PR001046 HCDR3 Chothia, PR004433 HCDR3 Chothia
RNYDDTRGTDVFDI

SEQ ID NO: 43 - protein, 8 aa, Artificial Sequence
  PR002129 HCDR3 Chothia
EQARSFDL

SEQ ID NO: 44 - protein, 16 aa, Artificial Sequence
  PR004432 HCDR3 Chothia
DNYYGSGSPPVDALDI

SEQ ID NO: 45 - protein, 11 aa, Artificial Sequence
  PR000020 HFWR4 Chothia, PR000184 HFWR4 Chothia, PR000759 HFWR4 Chothia
WGQGTMVTVSS

SEQ ID NO: 46 - protein, 11 aa, Artificial Sequence
  PR000453 HFWR4 Chothia
WGQGTQVTVSS

SEQ ID NO: 47 - protein, 11 aa, Artificial Sequence
  PR002129 HFWR4 Chothia
WGRGTLVTVSS

SEQ ID NO: 48 - protein, 23 aa, Artificial Sequence
  PR002129 LFWR1 Chothia
DIQLTQSPYSLSASVGDRVTITC

SEQ ID NO: 49 - protein, 11 aa, Artificial Sequence
  PR002129 LCDR1 Chothia
RASQTINNWLA

SEQ ID NO: 50 - protein, 15 aa, Artificial Sequence
  PR002129 LFWR2 Chothia
WYQQKPGKAPKLLIY

SEQ ID NO: 51 - protein, 7 aa, Artificial Sequence
  PR002129 LCDR2 Chothia
KASSLES

SEQ ID NO: 52 - protein, 32 aa, Artificial Sequence
  PR002129 LFWR3 Chothia
GVPSRFSGSGSGTEFTLTISSLQPDDFATYYC

SEQ ID NO: 53 - protein, 11 aa, Artificial Sequence
  PR002129 LCDR3 Chothia
QQYKLYSPMYT

SEQ ID NO: 54 - protein, 10 aa, Artificial Sequence
  PR002129 LFWR4 Chothia
FGQGTKVEIK

SEQ ID NO: 55 - protein, 118 aa, Artificial Sequence
  PR000020 VH
EVQLVETGGGLIQPGGSLRLSCAASGLNVSRHYLSWVRQAPGKGLEWVAVIYSGGGIEYVDSVKGRFTISRDNANNTLYLQMRSLRTEDSAVYYCARAIPRPHGSDIWGQGTMVTVSS

SEQ ID NO: 56 - protein, 119 aa, Artificial Sequence
  PR000184 VH
EVQLVESGGGLIQPGGSLRLSCAVSGFTVSKNYMSWVRQAPGKGLEWVSVVYSGGSKTYADSVKGRFTISRDNSKNTLYLQMNSLRAEDTAVYYCARAVPHSPSSFDIWGQGTMVTVSS

SEQ ID NO: 57 - protein, 118 aa, Artificial Sequence
  PR000453 VH
EVQLVESGGGLVQAGGSLRLSCAASGRTFTMGWFRQAPGKEREFVAAISLSPTLAYYAESVKGRFTISRDNAKNTVVLQMNSLKPEDTALYYCAADRKSVMSIRPDYWGQGTQVTVSS

SEQ ID NO: 58 - protein, 122 aa, Artificial Sequence
  PR000759 VH
EVQLVESGGGVVQPGRSLRLSCAASGFTFSSFAFHWVRQAPGKGLEGVAVIWYDGRNENYADSVKGRFTISRDNSKNMLYLQMNSLRAEDTAVYYCARGRGVLGDTRAFDIWGQGTMVTVSS

SEQ ID NO: 59 - protein, 122 aa, Artificial Sequence
  PR001046 VH
EVQLVETGGGLIQPGGSLRLSCAASGFTVSDNYMTWVRQAPGKGLEWVSVIFSGGNTYYADSVKGRFTISRDNAKNTLYLQMNSLRAEDTALYYCARRNYDDTRGTDVFDIWGQGTMVTVSS

SEQ ID NO: 60 - protein, 117 aa, Artificial Sequence
  PR002129 VH
QVQLVQSGGGVVQPGRSLRLSCAASGFTFSSYGMHWVRQAPGKGLEWVAVIWYDGSNKDYADSVKGRFTISRDTSKNTLYLQMNSLRAEDTAVYYCAREQARSFDLWGRGTLVTVSS

SEQ ID NO: 61 - protein, 128 aa, Artificial Sequence
  PR004432 VH
EVQLQQSGPGLVKPSQTLSLTCAISGDSVSNNYAAWNWIRQSPSRGLEWLGRTYYRSKWYNDYAVSVKSRITINPDTSKNQFSLQLNRVTPEDTAVYYCARDNYYGSGSPPVDALDIWGQGTMVTVSS

SEQ ID NO: 62 - protein, 122 aa, Artificial Sequence
  PR004433 VH
EVQLVETGGGLIQPGGSLRLSCAASGFTVSDSYMTWVRQAPGKGLEWVSVIFSGGRTYYSDSVKGRFTISRDNAKNTLYLQMNSLRAEDTALYYCARRNYDDTRGTDVFDIWGQGTMVTVSS

SEQ ID NO: 63 - protein, 109 aa, Artificial Sequence
  PR002129 VL
DIQLTQSPYSLSASVGDRVTITCRASQTINNWLAWYQQKPGKAPKLLIYKASSLESGVPSRFSGSGSGTEFTLTISSLQPDDFATYYCQQYKLYSPMYTFGQGTKVEIK

SEQ ID NO: 64 - protein, 351 aa, Artificial Sequence
  PR000020 HC
SEVQLVETGGGLIQPGGSLRLSCAASGLNVSRHYLSWVRQAPGKGLEWVAVIYSGGGIEYVDSVKGRFTISRDNANNTLYLQMRSLRTEDSAVYYCARAIPRPHGSDIWGQGTMVTVSSEPKSCDKTHTCPPCPAPELLGGPSVFLFPPKPKDTLMISRTPEVTCVVVDVSHEDPEVKFNWYVDGVEVHNAKTKPREEQYNSTYRVVSVLTVLHQDWLNGKEYKCKVSNKALPAPIEKTISKAKGQPREPQVYTLPPSREEMTKNQVSLTCLVKGFYPSDIAVEWESNGQPENNYKTTPPVLDSDGSFFLYSKLTVDKSRWQQGNVFSCSVMHEALHNHYTQKSLSLSPGK

SEQ ID NO: 65 - protein, 351 aa, Artificial Sequence
  PR000184 HC
EVQLVESGGGLIQPGGSLRLSCAVSGFTVSKNYMSWVRQAPGKGLEWVSVVYSGGSKTYADSVKGRFTISRDNSKNTLYLQMNSLRAEDTAVYYCARAVPHSPSSFDIWGQGTMVTVSSEPKSCDKTHTCPPCPAPELLGGPSVFLFPPKPKDTLMISRTPEVTCVVVDVSHEDPEVKFNWYVDGVEVHNAKTKPREEQYNSTYRVVSVLTVLHQDWLNGKEYKCKVSNKALPAPIEKTISKAKGQPREPQVYTLPPSREEMTKNQVSLTCLVKGFYPSDIAVEWESNGQPENNYKTTPPVLDSDGSFFLYSKLTVDKSRWQQGNVFSCSVMHEALHNHYTQKSLSLSPGK

SEQ ID NO: 66 - protein, 350 aa, Artificial Sequence
  PR000453 HC
EVQLVESGGGLVQAGGSLRLSCAASGRTFTMGWFRQAPGKEREFVAAISLSPTLAYYAESVKGRFTISRDNAKNTVVLQMNSLKPEDTALYYCAADRKSVMSIRPDYWGQGTQVTVSSEPKSCDKTHTCPPCPAPELLGGPSVFLFPPKPKDTLMISRTPEVTCVVVDVSHEDPEVKFNWYVDGVEVHNAKTKPREEQYNSTYRVVSVLTVLHQDWLNGKEYKCKVSNKALPAPIEKTISKAKGQPREPQVYTLPPSREEMTKNQVSLTCLVKGFYPSDIAVEWESNGQPENNYKTTPPVLDSDGSFFLYSKLTVDKSRWQQGNVFSCSVMHEALHNHYTQKSLSLSPGK

SEQ ID NO: 67 - protein, 354 aa, Artificial Sequence
  PR000759 HC
EVQLVESGGGVVQPGRSLRLSCAASGFTFSSFAFHWVRQAPGKGLEGVAVIWYDGRNENYADSVKGRFTISRDNSKNMLYLQMNSLRAEDTAVYYCARGRGVLGDTRAFDIWGQGTMVTVSSEPKSCDKTHTCPPCPAPELLGGPSVFLFPPKPKDTLMISRTPEVTCVVVDVSHEDPEVKFNWYVDGVEVHNAKTKPREEQYNSTYRVVSVLTVLHQDWLNGKEYKCKVSNKALPAPIEKTISKAKGQPREPQVYTLPPSREEMTKNQVSLTCLVKGFYPSDIAVEWESNGQPENNYKTTPPVLDSDGSFFLYSKLTVDKSRWQQGNVFSCSVMHEALHNHYTQKSLSLSPGK

SEQ ID NO: 68 - protein, 354 aa, Artificial Sequence
  PR001046 HC
EVQLVETGGGLIQPGGSLRLSCAASGFTVSDNYMTWVRQAPGKGLEWVSVIFSGGNTYYADSVKGRFTISRDNAKNTLYLQMNSLRAEDTALYYCARRNYDDTRGTDVFDIWGQGTMVTVSSEPKSCDKTHTCPPCPAPELLGGPSVFLFPPKPKDTLMISRTPEVTCVVVDVSHEDPEVKFNWYVDGVEVHNAKTKPREEQYNSTYRVVSVLTVLHQDWLNGKEYKCKVSNKALPAPIEKTISKAKGQPREPQVYTLPPSREEMTKNQVSLTCLVKGFYPSDIAVEWESNGQPENNYKTTPPVLDSDGSFFLYSKLTVDKSRWQQGNVFSCSVMHEALHNHYTQKSLSLSPGK

SEQ ID NO: 69 - protein, 360 aa, Artificial Sequence
  PR004432 HC
EVQLQQSGPGLVKPSQTLSLTCAISGDSVSNNYAAWNWIRQSPSRGLEWLGRTYYRSKWYNDYAVSVKSRITINPDTSKNQFSLQLNRVTPEDTAVYYCARDNYYGSGSPPVDALDIWGQGTMVTVSSEPKSCDKTHTCPPCPAPELLGGPSVFLFPPKPKDTLMISRTPEVTCVVVDVSHEDPEVKFNWYVDGVEVHNAKTKPREEQYNSTYRVVSVLTVLHQDWLNGKEYKCKVSNKALPAPIEKTISKAKGQPREPQVYTLPPSREEMTKNQVSLTCLVKGFYPSDIAVEWESNGQPENNYKTTPPVLDSDGSFFLYSKLTVDKSRWQQGNVFSCSVMHEALHNHYTQKSLSLSPGK

SEQ ID NO: 70 - protein, 354 aa, Artificial Sequence
  PR004433 HC
EVQLVETGGGLIQPGGSLRLSCAASGFTVSDSYMTWVRQAPGKGLEWVSVIFSGGRTYYSDSVKGRFTISRDNAKNTLYLQMNSLRAEDTALYYCARRNYDDTRGTDVFDIWGQGTMVTVSSEPKSCDKTHTCPPCPAPELLGGPSVFLFPPKPKDTLMISRTPEVTCVVVDVSHEDPEVKFNWYVDGVEVHNAKTKPREEQYNSTYRVVSVLTVLHQDWLNGKEYKCKVSNKALPAPIEKTISKAKGQPREPQVYTLPPSREEMTKNQVSLTCLVKGFYPSDIAVEWESNGQPENNYKTTPPVLDSDGSFFLYSKLTVDKSRWQQGNVFSCSVMHEALHNHYTQKSLSLSPGK

SEQ ID NO: 71 - protein, 478 aa, Artificial Sequence
  PR002129 SCFV
QVQLVQSGGGVVQPGRSLRLSCAASGFTFSSYGMHWVRQAPGKGLEWVAVIWYDGSNKDYADSVKGRFTISRDTSKNTLYLQMNSLRAEDTAVYYCAREQARSFDLWGRGTLVTVSSGGGGSGGGGSGGGGSDIQLTQSPYSLSASVGDRVTITCRASQTINNWLAWYQQKPGKAPKLLIYKASSLESGVPSRFSGSGSGTEFTLTISSLQPDDFATYYCQQYKLYSPMYTFGQGTKVEIKGGGASEPKSCDKTHTCPPCPAPELLGGPSVFLFPPKPKDTLMISRTPEVTCVVVDVSHEDPEVKFNWYVDGVEVHNAKTKPREEQYNSTYRVVSVLTVLHQDWLNGKEYKCKVSNKALPAPIEKTISKAKGQPREPQVYTLPPSREEMTKNQVSLTCLVKGFYPSDIAVEWESNGQPENNYKTTPPVLDSDGSFFLYSKLTVDKSRWQQGNVFSCSVMHEALHNHYTQKSLSLSPGK

SEQ ID NO: 72 - protein, 232 aa, Homo sapiens
  Human IgG1 Fc (comprising a hinge region)
EPKSCDKTHTCPPCPAPELLGGPSVFLFPPKPKDTLMISRTPEVTCVVVDVSHEDPEVKFNWYVDGVEVHNAKTKPREEQYNSTYRVVSVLTVLHQDWLNGKEYKCKVSNKALPAPIEKTISKAKGQPREPQVYTLPPSREEMTKNQVSLTCLVKGFYPSDIAVEWESNGQPENNYKTTPPVLDSDGSFFLYSKLTVDKSRWQQGNVFSCSVMHEALHNHYTQKSLSLSPGK

SEQ ID NO: 73 - protein, 15 aa, Homo sapiens
  Human IgG1 hinge region
EPKSCDKTHTCPPCP

SEQ ID NO: 74 - protein, 13 aa, Artificial Sequence
  Human IgG1 hinge region var. C220-X3
  misc_feature (6)..(8): Xaa can be any natural amino acid
EPKSCXXXCPPCP

SEQ ID NO: 75 - protein, 14 aa, Artificial Sequence
  Human IgG1 hinge region var. C220-X4
  misc_feature (6)..(9): Xaa can be any natural amino acid
EPKSCXXXXCPPCP

SEQ ID NO: 76 - protein, 15 aa, Artificial Sequence
  Human IgG1 hinge region var. C220-X5
  misc_feature (6)..(10): Xaa can be any natural amino acid
EPKSCXXXXXCPPCP

SEQ ID NO: 77 - protein, 16 aa, Artificial Sequence
  Human IgG1 hinge region var. C220-X6
  misc_feature (6)..(11): Xaa can be any natural amino acid
EPKSCXXXXXXCPPCP

SEQ ID NO: 78 - protein, 17 aa, Artificial Sequence
  Human IgG1 hinge region var. C220-X7
  misc_feature (6)..(12): Xaa can be any natural amino acid
EPKSCXXXXXXXCPPCP

SEQ ID NO: 79 - protein, 18 aa, Artificial Sequence
  Human IgG1 hinge region var. C220-X8
  misc_feature (6)..(13): Xaa can be any natural amino acid
EPKSCXXXXXXXXCPPCP

SEQ ID NO: 80 - protein, 19 aa, Artificial Sequence
  Human IgG1 hinge region var. C220-X9
  misc_feature (6)..(14): Xaa can be any natural amino acid
EPKSCXXXXXXXXXCPPCP

SEQ ID NO: 81 - protein, 20 aa, Artificial Sequence
  Human IgG1 hinge region var. C220-X10
  misc_feature (6)..(15): Xaa can be any natural amino acid
EPKSCXXXXXXXXXXCPPCP

SEQ ID NO: 82 - protein, 13 aa, Artificial Sequence
  Hinge3_5
EPKSCQPRCPPCP

SEQ ID NO: 83 - protein, 13 aa, Artificial Sequence
  Hinge3_6
EPKSCAGWCPPCP

SEQ ID NO: 84 - protein, 13 aa, Artificial Sequence
  Hinge3_18
EPKSCNVACPPCP

SEQ ID NO: 85 - protein, 14 aa, Artificial Sequence
  Hinge4_1
EPKSCTGKMCPPCP

SEQ ID NO: 86 - protein, 14 aa, Artificial Sequence
  Hinge4_6
EPKSCRDARCPPCP

SEQ ID NO: 87 - protein, 14 aa, Artificial Sequence
  Hinge4_15
EPKSCRGTLCPPCP

SEQ ID NO: 88 - protein, 15 aa, Artificial Sequence
  Hinge5_2
EPKSCQAESRCPPCP

SEQ ID NO: 89 - protein, 15 aa, Artificial Sequence
  Hinge5_12
EPKSCKDYGRCPPCP

SEQ ID NO: 90 - protein, 15 aa, Artificial Sequence
  Hinge5_13
EPKSCSDNHDCPPCP

SEQ ID NO: 91 - protein, 16 aa, Artificial Sequence
  Hinge6_4
EPKSCAPVRPWCPPCP

SEQ ID NO: 92 - protein, 16 aa, Artificial Sequence
  Hinge6_15
EPKSCSGPSTLCPPCP

SEQ ID NO: 93 - protein, 16 aa, Artificial Sequence
  Hinge6_18
EPKSCSAVPRRCPPCP

SEQ ID NO: 94 - protein, 17 aa, Artificial Sequence
  Hinge7_2
EPKSCAVLPEIGCPPCP

SEQ ID NO: 95 - protein, 17 aa, Artificial Sequence
  Hinge7_3
EPKSCWLYISDKCPPCP

SEQ ID NO: 96 - protein, 17 aa, Artificial Sequence
  Hinge7_19
EPKSCSYLFGRVCPPCP

SEQ ID NO: 97 - protein, 18 aa, Artificial Sequence
  Hinge8_8
EPKSCMPRLLFHSCPPCP

SEQ ID NO: 98 - protein, 18 aa, Artificial Sequence
  Hinge8_18
EPKSCSSDVVGGRCPPCP

SEQ ID NO: 99 - protein, 18 aa, Artificial Sequence
  Hinge8_20
EPKSCRMTVYGSRCPPCP

SEQ ID NO: 100 - protein, 19 aa, Artificial Sequence
  Hinge9_5
EPKSCLALPGVMSPCPPCP

SEQ ID NO: 101 - protein, 19 aa, Artificial Sequence
  Hinge9_7
EPKSCASMNRGGGGCPPCP

SEQ ID NO: 102 - protein, 19 aa, Artificial Sequence
  Hinge9_14
EPKSCGGGPFLWLVCPPCP

SEQ ID NO: 103 - protein, 20 aa, Artificial Sequence
  Hinge10_3
EPKSCQMSVFARHFPCPPCP

SEQ ID NO: 104 - protein, 20 aa, Artificial Sequence
  Hinge10_5
EPKSCSVGRFGSMLECPPCP

SEQ ID NO: 105 - protein, 20 aa, Artificial Sequence
  Hinge10_7
EPKSCITEWSVRDLQCPPCP

SEQ ID NO: 106 - protein, 352 aa, Artificial Sequence
  PR006031 chain
EVQLVETGGGLIQPGGSLRLSCAASGFTVSDSYMTWVRQAPGKGLEWVSVIFSGGRTYYSDSVKGRFTISRDNAKNTLYLQMNSLRAEDTALYYCARRNYDDTRGTDVFDIWGQGTMVTVSSEPKSCQPRCPPCPAPELLGGPSVFLFPPKPKDTLMISRTPEVTCVVVDVSHEDPEVKFNWYVDGVEVHNAKTKPREEQYNSTYRVVSVLTVLHQDWLNGKEYKCKVSNKALPAPIEKTISKAKGQPREPQVYTLPPSREEMTKNQVSLTCLVKGFYPSDIAVEWESNGQPENNYKTTPPVLDSDGSFFLYSKLTVDKSRWQQGNVFSCSVMHEALHNHYTQKSLSLSPGK

SEQ ID NO: 107 - protein, 352 aa, Artificial Sequence
  PR006032 chain
EVQLVETGGGLIQPGGSLRLSCAASGFTVSDSYMTWVRQAPGKGLEWVSVIFSGGRTYYSDSVKGRFTISRDNAKNTLYLQMNSLRAEDTALYYCARRNYDDTRGTDVFDIWGQGTMVTVSSEPKSCAGWCPPCPAPELLGGPSVFLFPPKPKDTLMISRTPEVTCVVVDVSHEDPEVKFNWYVDGVEVHNAKTKPREEQYNSTYRVVSVLTVLHQDWLNGKEYKCKVSNKALPAPIEKTISKAKGQPREPQVYTLPPSREEMTKNQVSLTCLVKGFYPSDIAVEWESNGQPENNYKTTPPVLDSDGSFFLYSKLTVDKSRWQQGNVFSCSVMHEALHNHYTQKSLSLSPGK

SEQ ID NO: 108 - protein, 352 aa, Artificial Sequence
  PR006033 chain
EVQLVETGGGLIQPGGSLRLSCAASGFTVSDSYMTWVRQAPGKGLEWVSVIFSGGRTYYSDSVKGRFTISRDNAKNTLYLQMNSLRAEDTALYYCARRNYDDTRGTDVFDIWGQGTMVTVSSEPKSCNVACPPCPAPELLGGPSVFLFPPKPKDTLMISRTPEVTCVVVDVSHEDPEVKFNWYVDGVEVHNAKTKPREEQYNSTYRVVSVLTVLHQDWLNGKEYKCKVSNKALPAPIEKTISKAKGQPREPQVYTLPPSREEMTKNQVSLTCLVKGFYPSDIAVEWESNGQPENNYKTTPPVLDSDGSFFLYSKLTVDKSRWQQGNVFSCSVMHEALHNHYTQKSLSLSPGK

SEQ ID NO: 109 - protein, 353 aa, Artificial Sequence
  PR006034 chain
EVQLVETGGGLIQPGGSLRLSCAASGFTVSDSYMTWVRQAPGKGLEWVSVIFSGGRTYYSDSVKGRFTISRDNAKNTLYLQMNSLRAEDTALYYCARRNYDDTRGTDVFDIWGQGTMVTVSSEPKSCTGKMCPPCPAPELLGGPSVFLFPPKPKDTLMISRTPEVTCVVVDVSHEDPEVKFNWYVDGVEVHNAKTKPREEQYNSTYRVVSVLTVLHQDWLNGKEYKCKVSNKALPAPIEKTISKAKGQPREPQVYTLPPSREEMTKNQVSLTCLVKGFYPSDIAVEWESNGQPENNYKTTPPVLDSDGSFFLYSKLTVDKSRWQQGNVFSCSVMHEALHNHYTQKSLSLSPGK

SEQ ID NO: 110 - protein, 353 aa, Artificial Sequence
  PR006035 chain
EVQLVETGGGLIQPGGSLRLSCAASGFTVSDSYMTWVRQAPGKGLEWVSVIFSGGRTYYSDSVKGRFTISRDNAKNTLYLQMNSLRAEDTALYYCARRNYDDTRGTDVFDIWGQGTMVTVSSEPKSCRDARCPPCPAPELLGGPSVFLFPPKPKDTLMISRTPEVTCVVVDVSHEDPEVKFNWYVDGVEVHNAKTKPREEQYNSTYRVVSVLTVLHQDWLNGKEYKCKVSNKALPAPIEKTISKAKGQPREPQVYTLPPSREEMTKNQVSLTCLVKGFYPSDIAVEWESNGQPENNYKTTPPVLDSDGSFFLYSKLTVDKSRWQQGNVFSCSVMHEALHNHYTQKSLSLSPGK

SEQ ID NO: 111 - protein, 353 aa, Artificial Sequence
  PR006036 chain
EVQLVETGGGLIQPGGSLRLSCAASGFTVSDSYMTWVRQAPGKGLEWVSVIFSGGRTYYSDSVKGRFTISRDNAKNTLYLQMNSLRAEDTALYYCARRNYDDTRGTDVFDIWGQGTMVTVSSEPKSCRGTLCPPCPAPELLGGPSVFLFPPKPKDTLMISRTPEVTCVVVDVSHEDPEVKFNWYVDGVEVHNAKTKPREEQYNSTYRVVSVLTVLHQDWLNGKEYKCKVSNKALPAPIEKTISKAKGQPREPQVYTLPPSREEMTKNQVSLTCLVKGFYPSDIAVEWESNGQPENNYKTTPPVLDSDGSFFLYSKLTVDKSRWQQGNVFSCSVMHEALHNHYTQKSLSLSPGK

SEQ ID NO: 112 - protein, 354 aa, Artificial Sequence
  PR006037 chain
EVQLVETGGGLIQPGGSLRLSCAASGFTVSDSYMTWVRQAPGKGLEWVSVIFSGGRTYYSDSVKGRFTISRDNAKNTLYLQMNSLRAEDTALYYCARRNYDDTRGTDVFDIWGQGTMVTVSSEPKSCQAESRCPPCPAPELLGGPSVFLFPPKPKDTLMISRTPEVTCVVVDVSHEDPEVKFNWYVDGVEVHNAKTKPREEQYNSTYRVVSVLTVLHQDWLNGKEYKCKVSNKALPAPIEKTISKAKGQPREPQVYTLPPSREEMTKNQVSLTCLVKGFYPSDIAVEWESNGQPENNYKTTPPVLDSDGSFFLYSKLTVDKSRWQQGNVFSCSVMHEALHNHYTQKSLSLSPGK

SEQ ID NO: 113 - protein, 354 aa, Artificial Sequence
  PR006038 chain
EVQLVETGGGLIQPGGSLRLSCAASGFTVSDSYMTWVRQAPGKGLEWVSVIFSGGRTYYSDSVKGRFTISRDNAKNTLYLQMNSLRAEDTALYYCARRNYDDTRGTDVFDIWGQGTMVTVSSEPKSCKDYGRCPPCPAPELLGGPSVFLFPPKPKDTLMISRTPEVTCVVVDVSHEDPEVKFNWYVDGVEVHNAKTKPREEQYNSTYRVVSVLTVLHQDWLNGKEYKCKVSNKALPAPIEKTISKAKGQPREPQVYTLPPSREEMTKNQVSLTCLVKGFYPSDIAVEWESNGQPENNYKTTPPVLDSDGSFFLYSKLTVDKSRWQQGNVFSCSVMHEALHNHYTQKSLSLSPGK

SEQ ID NO: 114 - protein, 354 aa, Artificial Sequence
  PR006039 chain
EVQLVETGGGLIQPGGSLRLSCAASGFTVSDSYMTWVRQAPGKGLEWVSVIFSGGRTYYSDSVKGRFTISRDNAKNTLYLQMNSLRAEDTALYYCARRNYDDTRGTDVFDIWGQGTMVTVSSEPKSCSDNHDCPPCPAPELLGGPSVFLFPPKPKDTLMISRTPEVTCVVVDVSHEDPEVKFNWYVDGVEVHNAKTKPREEQYNSTYRVVSVLTVLHQDWLNGKEYKCKVSNKALPAPIEKTISKAKGQPREPQVYTLPPSREEMTKNQVSLTCLVKGFYPSDIAVEWESNGQPENNYKTTPPVLDSDGSFFLYSKLTVDKSRWQQGNVFSCSVMHEALHNHYTQKSLSLSPGK

SEQ ID NO: 115 - protein, 355 aa, Artificial Sequence
  PR006040 chain
EVQLVETGGGLIQPGGSLRLSCAASGFTVSDSYMTWVRQAPGKGLEWVSVIFSGGRTYYSDSVKGRFTISRDNAKNTLYLQMNSLRAEDTALYYCARRNYDDTRGTDVFDIWGQGTMVTVSSEPKSCAPVRPWCPPCPAPELLGGPSVFLFPPKPKDTLMISRTPEVTCVVVDVSHEDPEVKFNWYVDGVEVHNAKTKPREEQYNSTYRVVSVLTVLHQDWLNGKEYKCKVSNKALPAPIEKTISKAKGQPREPQVYTLPPSREEMTKNQVSLTCLVKGFYPSDIAVEWESNGQPENNYKTTPPVLDSDGSFFLYSKLTVDKSRWQQGNVFSCSVMHEALHNHYTQKSLSLSPGK

SEQ ID NO: 116 - protein, 355 aa, Artificial Sequence
  PR006041 chain
EVQLVETGGGLIQPGGSLRLSCAASGFTVSDSYMTWVRQAPGKGLEWVSVIFSGGRTYYSDSVKGRFTISRDNAKNTLYLQMNSLRAEDTALYYCARRNYDDTRGTDVFDIWGQGTMVTVSSEPKSCSGPSTLCPPCPAPELLGGPSVFLFPPKPKDTLMISRTPEVTCVVVDVSHEDPEVKFNWYVDGVEVHNAKTKPREEQYNSTYRVVSVLTVLHQDWLNGKEYKCKVSNKALPAPIEKTISKAKGQPREPQVYTLPPSREEMTKNQVSLTCLVKGFYPSDIAVEWESNGQPENNYKTTPPVLDSDGSFFLYSKLTVDKSRWQQGNVFSCSVMHEALHNHYTQKSLSLSPGK

SEQ ID NO: 117 - protein, 355 aa, Artificial Sequence
  PR006042 chain
EVQLVETGGGLIQPGGSLRLSCAASGFTVSDSYMTWVRQAPGKGLEWVSVIFSGGRTYYSDSVKGRFTISRDNAKNTLYLQMNSLRAEDTALYYCARRNYDDTRGTDVFDIWGQGTMVTVSSEPKSCSAVPRRCPPCPAPELLGGPSVFLFPPKPKDTLMISRTPEVTCVVVDVSHEDPEVKFNWYVDGVEVHNAKTKPREEQYNSTYRVVSVLTVLHQDWLNGKEYKCKVSNKALPAPIEKTISKAKGQPREPQVYTLPPSREEMTKNQVSLTCLVKGFYPSDIAVEWESNGQPENNYKTTPPVLDSDGSFFLYSKLTVDKSRWQQGNVFSCSVMHEALHNHYTQKSLSLSPGK

SEQ ID NO: 118 - protein, 356 aa, Artificial Sequence
  PR006310 chain
EVQLVETGGGLIQPGGSLRLSCAASGFTVSDSYMTWVRQAPGKGLEWVSVIFSGGRTYYSDSVKGRFTISRDNAKNTLYLQMNSLRAEDTALYYCARRNYDDTRGTDVFDIWGQGTMVTVSSEPKSCAVLPEIGCPPCPAPELLGGPSVFLFPPKPKDTLMISRTPEVTCVVVDVSHEDPEVKFNWYVDGVEVHNAKTKPREEQYNSTYRVVSVLTVLHQDWLNGKEYKCKVSNKALPAPIEKTISKAKGQPREPQVYTLPPSREEMTKNQVSLTCLVKGFYPSDIAVEWESNGQPENNYKTTPPVLDSDGSFFLYSKLTVDKSRWQQGNVFSCSVMHEALHNHYTQKSLSLSPGK

SEQ ID NO: 119 - protein, 356 aa, Artificial Sequence
  PR006311 chain
EVQLVETGGGLIQPGGSLRLSCAASGFTVSDSYMTWVRQAPGKGLEWVSVIFSGGRTYYSDSVKGRFTISRDNAKNTLYLQMNSLRAEDTALYYCARRNYDDTRGTDVFDIWGQGTMVTVSSEPKSCWLYISDKCPPCPAPELLGGPSVFLFPPKPKDTLMISRTPEVTCVVVDVSHEDPEVKFNWYVDGVEVHNAKTKPREEQYNSTYRVVSVLTVLHQDWLNGKEYKCKVSNKALPAPIEKTISKAKGQPREPQVYTLPPSREEMTKNQVSLTCLVKGFYPSDIAVEWESNGQPENNYKTTPPVLDSDGSFFLYSKLTVDKSRWQQGNVFSCSVMHEALHNHYTQKSLSLSPGK

SEQ ID NO: 120 - protein, 356 aa, Artificial Sequence
  PR006312 chain
EVQLVETGGGLIQPGGSLRLSCAASGFTVSDSYMTWVRQAPGKGLEWVSVIFSGGRTYYSDSVKGRFTISRDNAKNTLYLQMNSLRAEDTALYYCARRNYDDTRGTDVFDIWGQGTMVTVSSEPKSCSYLFGRVCPPCPAPELLGGPSVFLFPPKPKDTLMISRTPEVTCVVVDVSHEDPEVKFNWYVDGVEVHNAKTKPREEQYNSTYRVVSVLTVLHQDWLNGKEYKCKVSNKALPAPIEKTISKAKGQPREPQVYTLPPSREEMTKNQVSLTCLVKGFYPSDIAVEWESNGQPENNYKTTPPVLDSDGSFFLYSKLTVDKSRWQQGNVFSCSVMHEALHNHYTQKSLSLSPGK

SEQ ID NO: 121 - protein, 357 aa, Artificial Sequence
  PR006313 chain
EVQLVETGGGLIQPGGSLRLSCAASGFTVSDSYMTWVRQAPGKGLEWVSVIFSGGRTYYSDSVKGRFTISRDNAKNTLYLQMNSLRAEDTALYYCARRNYDDTRGTDVFDIWGQGTMVTVSSEPKSCMPRLLFHSCPPCPAPELLGGPSVFLFPPKPKDTLMISRTPEVTCVVVDVSHEDPEVKFNWYVDGVEVHNAKTKPREEQYNSTYRVVSVLTVLHQDWLNGKEYKCKVSNKALPAPIEKTISKAKGQPREPQVYTLPPSREEMTKNQVSLTCLVKGFYPSDIAVEWESNGQPENNYKTTPPVLDSDGSFFLYSKLTVDKSRWQQGNVFSCSVMHEALHNHYTQKSLSLSPGK

SEQ ID NO: 122 - protein, 357 aa, Artificial Sequence
  PR006314 chain
EVQLVETGGGLIQPGGSLRLSCAASGFTVSDSYMTWVRQAPGKGLEWVSVIFSGGRTYYSDSVKGRFTISRDNAKNTLYLQMNSLRAEDTALYYCARRNYDDTRGTDVFDIWGQGTMVTVSSEPKSCSSDVVGGRCPPCPAPELLGGPSVFLFPPKPKDTLMISRTPEVTCVVVDVSHEDPEVKFNWYVDGVEVHNAKTKPREEQYNSTYRVVSVLTVLHQDWLNGKEYKCKVSNKALPAPIEKTISKAKGQPREPQVYTLPPSREEMTKNQVSLTCLVKGFYPSDIAVEWESNGQPENNYKTTPPVLDSDGSFFLYSKLTVDKSRWQQGNVFSCSVMHEALHNHYTQKSLSLSPGK

SEQ ID NO: 123 - protein, 357 aa, Artificial Sequence
  PR006315 chain
EVQLVETGGGLIQPGGSLRLSCAASGFTVSDSYMTWVRQAPGKGLEWVSVIFSGGRTYYSDSVKGRFTISRDNAKNTLYLQMNSLRAEDTALYYCARRNYDDTRGTDVFDIWGQGTMVTVSSEPKSCRMTVYGSRCPPCPAPELLGGPSVFLFPPKPKDTLMISRTPEVTCVVVDVSHEDPEVKFNWYVDGVEVHNAKTKPREEQYNSTYRVVSVLTVLHQDWLNGKEYKCKVSNKALPAPIEKTISKAKGQPREPQVYTLPPSREEMTKNQVSLTCLVKGFYPSDIAVEWESNGQPENNYKTTPPVLDSDGSFFLYSKLTVDKSRWQQGNVFSCSVMHEALHNHYTQKSLSLSPGK

SEQ ID NO: 124 - protein, 358 aa, Artificial Sequence
  PR006316 chain
EVQLVETGGGLIQPGGSLRLSCAASGFTVSDSYMTWVRQAPGKGLEWVSVIFSGGRTYYSDSVKGRFTISRDNAKNTLYLQMNSLRAEDTALYYCARRNYDDTRGTDVFDIWGQGTMVTVSSEPKSCLALPGVMSPCPPCPAPELLGGPSVFLFPPKPKDTLMISRTPEVTCVVVDVSHEDPEVKFNWYVDGVEVHNAKTKPREEQYNSTYRVVSVLTVLHQDWLNGKEYKCKVSNKALPAPIEKTISKAKGQPREPQVYTLPPSREEMTKNQVSLTCLVKGFYPSDIAVEWESNGQPENNYKTTPPVLDSDGSFFLYSKLTVDKSRWQQGNVFSCSVMHEALHNHYTQKSLSLSPGK

SEQ ID NO: 125 - protein, 358 aa, Artificial Sequence
  PR006317 chain
EVQLVETGGGLIQPGGSLRLSCAASGFTVSDSYMTWVRQAPGKGLEWVSVIFSGGRTYYSDSVKGRFTISRDNAKNTLYLQMNSLRAEDTALYYCARRNYDDTRGTDVFDIWGQGTMVTVSSEPKSCASMNRGGGGCPPCPAPELLGGPSVFLFPPKPKDTLMISRTPEVTCVVVDVSHEDPEVKFNWYVDGVEVHNAKTKPREEQYNSTYRVVSVLTVLHQDWLNGKEYKCKVSNKALPAPIEKTISKAKGQPREPQVYTLPPSREEMTKNQVSLTCLVKGFYPSDIAVEWESNGQPENNYKTTPPVLDSDGSFFLYSKLTVDKSRWQQGNVFSCSVMHEALHNHYTQKSLSLSPGK

SEQ ID NO: 126 - protein, 358 aa, Artificial Sequence
  PR006318 chain
EVQLVETGGGLIQPGGSLRLSCAASGFTVSDSYMTWVRQAPGKGLEWVSVIFSGGRTYYSDSVKGRFTISRDNAKNTLYLQMNSLRAEDTALYYCARRNYDDTRGTDVFDIWGQGTMVTVSSEPKSCGGGPFLWLVCPPCPAPELLGGPSVFLFPPKPKDTLMISRTPEVTCVVVDVSHEDPEVKFNWYVDGVEVHNAKTKPREEQYNSTYRVVSVLTVLHQDWLNGKEYKCKVSNKALPAPIEKTISKAKGQPREPQVYTLPPSREEMTKNQVSLTCLVKGFYPSDIAVEWESNGQPENNYKTTPPVLDSDGSFFLYSKLTVDKSRWQQGNVFSCSVMHEALHNHYTQKSLSLSPGK

SEQ ID NO: 127 - protein, 359 aa, Artificial Sequence
  PR006319 chain
EVQLVETGGGLIQPGGSLRLSCAASGFTVSDSYMTWVRQAPGKGLEWVSVIFSGGRTYYSDSVKGRFTISRDNAKNTLYLQMNSLRAEDTALYYCARRNYDDTRGTDVFDIWGQGTMVTVSSEPKSCQMSVFARHFPCPPCPAPELLGGPSVFLFPPKPKDTLMISRTPEVTCVVVDVSHEDPEVKFNWYVDGVEVHNAKTKPREEQYNSTYRVVSVLTVLHQDWLNGKEYKCKVSNKALPAPIEKTISKAKGQPREPQVYTLPPSREEMTKNQVSLTCLVKGFYPSDIAVEWESNGQPENNYKTTPPVLDSDGSFFLYSKLTVDKSRWQQGNVFSCSVMHEALHNHYTQKSLSLSPGK

SEQ ID NO: 128 - protein, 359 aa, Artificial Sequence
  PR006320 chain
EVQLVETGGGLIQPGGSLRLSCAASGFTVSDSYMTWVRQAPGKGLEWVSVIFSGGRTYYSDSVKGRFTISRDNAKNTLYLQMNSLRAEDTALYYCARRNYDDTRGTDVFDIWGQGTMVTVSSEPKSCSVGRFGSMLECPPCPAPELLGGPSVFLFPPKPKDTLMISRTPEVTCVVVDVSHEDPEVKFNWYVDGVEVHNAKTKPREEQYNSTYRVVSVLTVLHQDWLNGKEYKCKVSNKALPAPIEKTISKAKGQPREPQVYTLPPSREEMTKNQVSLTCLVKGFYPSDIAVEWESNGQPENNYKTTPPVLDSDGSFFLYSKLTVDKSRWQQGNVFSCSVMHEALHNHYTQKSLSLSPGK

SEQ ID NO: 129 - protein, 359 aa, Artificial Sequence
  PR006321 chain
EVQLVETGGGLIQPGGSLRLSCAASGFTVSDSYMTWVRQAPGKGLEWVSVIFSGGRTYYSDSVKGRFTISRDNAKNTLYLQMNSLRAEDTALYYCARRNYDDTRGTDVFDIWGQGTMVTVSSEPKSCITEWSVRDLQCPPCPAPELLGGPSVFLFPPKPKDTLMISRTPEVTCVVVDVSHEDPEVKFNWYVDGVEVHNAKTKPREEQYNSTYRVVSVLTVLHQDWLNGKEYKCKVSNKALPAPIEKTISKAKGQPREPQVYTLPPSREEMTKNQVSLTCLVKGFYPSDIAVEWESNGQPENNYKTTPPVLDSDGSFFLYSKLTVDKSRWQQGNVFSCSVMHEALHNHYTQKSLSLSPGK

SEQ ID NO: 130 - protein, 128 aa, Artificial Sequence
  PR000892 VH
QVQLVESGGGVVQPGRSLRLSCAATGFTFSSYGMYWVRQAPGKGLEWVAAIWNDGSNNYYADSVKGRFTISRDDSKNTLNLQMNSLRAEDTAMYYCARDRLPMASLRYFDWLGVMDAWGQGTSVTVSS

SEQ ID NO: 131 - protein, 107 aa, Artificial Sequence
  PR000892 VL
DIQMTQSPSTLSASVGDRVTITCRASQSISSWLAWYQQKPGKAPKLLIYKASSLESGVPSRFSGSGSGTEFTLTISSLQTDDFATYYCQQYNSYLFTFGQGTKLEIK

SEQ ID NO: 132 - protein, 458 aa, Artificial Sequence
  PR000892 HC
QVQLVESGGGVVQPGRSLRLSCAATGFTFSSYGMYWVRQAPGKGLEWVAAIWNDGSNNYYADSVKGRFTISRDDSKNTLNLQMNSLRAEDTAMYYCARDRLPMASLRYFDWLGVMDAWGQGTSVTVSSASTKGPSVFPLAPSSKSTSGGTAALGCLVKDYFPEPVTVSWNSGALTSGVHTFPAVLQSSGLYSLSSVVTVPSSSLGTQTYICNVNHKPSNTKVDKKVEPKSCDKTHTCPPCPAPELLGGPSVFLFPPKPKDTLMISRTPEVTCVVVDVSHEDPEVKFNWYVDGVEVHNAKTKPREEQYNSTYRVVSVLTVLHQDWLNGKEYKCKVSNKALPAPIEKTISKAKGQPREPQVYTLPPSREEMTKNQVSLTCLVKGFYPSDIAVEWESNGQPENNYKTTPPVLDSDGSFFLYSKLTVDKSRWQQGNVFSCSVMHEALHNHYTQKSLSLSPGK

SEQ ID NO: 133 - protein, 214 aa, Artificial Sequence
  PR000892 LC
DIQMTQSPSTLSASVGDRVTITCRASQSISSWLAWYQQKPGKAPKLLIYKASSLESGVPSRFSGSGSGTEFTLTISSLQTDDFATYYCQQYNSYLFTFGQGTKLEIKRTVAAPSVFIFPPSDEQLKSGTASVVCLLNNFYPREAKVQWKVDNALQSGNSQESVTEQDSKDSTYSLSSTLTLSKADYEKHKVYACEVTHQGLSSPVTKSFNRGEC

SEQ ID NO: 134 - protein, 231 aa, Artificial Sequence
  PR005744 chain
QVQLVESGGGVVQPGRSLRLSCAATGFTFSSYGMYWVRQAPGKGLEWVAAIWNDGSNNYYADSVKGRFTISRDDSKNTLNLQMNSLRAEDTAMYYCARDRLPMASLRYFDWLGVMDAWGQGTSVTVSSASTKGPSVFPLAPSSKSTSGGTAALGCLVKDYFPEPVTVSWNSGALTSGVHTFPAVLQSSGLYSLSSVVTVPSSSLGTQTYICNVNHKPSNTKVDKKVEPKSC

SEQ ID NO: 135 - protein, 568 aa, Artificial Sequence
  PR005744 chain
DIQMTQSPSTLSASVGDRVTITCRASQSISSWLAWYQQKPGKAPKLLIYKASSLESGVPSRFSGSGSGTEFTLTISSLQTDDFATYYCQQYNSYLFTFGQGTKLEIKRTVAAPSVFIFPPSDEQLKSGTASVVCLLNNFYPREAKVQWKVDNALQSGNSQESVTEQDSKDSTYSLSSTLTLSKADYEKHKVYACEVTHQGLSSPVTKSFNRGECEVQLVETGGGLIQPGGSLRLSCAASGFTVSDSYMTWVRQAPGKGLEWVSVIFSGGRTYYSDSVKGRFTISRDNAKNTLYLQMNSLRAEDTALYYCARRNYDDTRGTDVFDIWGQGTMVTVSSEPKSCDKTHTCPPCPAPELLGGPSVFLFPPKPKDTLMISRTPEVTCVVVDVSHEDPEVKFNWYVDGVEVHNAKTKPREEQYNSTYRVVSVLTVLHQDWLNGKEYKCKVSNKALPAPIEKTISKAKGQPREPQVYTLPPSREEMTKNQVSLTCLVKGFYPSDIAVEWESNGQPENNYKTTPPVLDSDGSFFLYSKLTVDKSRWQQGNVFSCSVMHEALHNHYTQKSLSLSPGK

SEQ ID NO: 136 - DNA, 73 bp, Artificial Sequence
  Forward primer-3
  misc_feature (36)..(37): n is a, c, g or t
  misc_feature (39)..(40): n is a, c, g or t
  misc_feature (42)..(43): n is a, c, g or t
attaggtcaccgtctcctcagagcccaaatcttgtnnknnknnktgcccaccgtgcccagcacctgaactcct

SEQ ID NO: 137 - DNA, 76 bp, Artificial Sequence
  Forward primer-4
  misc_feature (36)..(37): n is a, c, g or t
  misc_feature (39)..(40): n is a, c, g or t
  misc_feature (42)..(43): n is a, c, g or t
  misc_feature (45)..(46): n is a, c, g or t
attaggtcaccgtctcctcagagcccaaatcttgtnnknnknnknnktgcccaccgtgcccagcacctgaactcct

SEQ ID NO: 138 - DNA, 79 bp, Artificial Sequence
  Forward primer-5
  misc_feature (36)..(37): n is a, c, g or t
  misc_feature (39)..(40): n is a, c, g or t
  misc_feature (42)..(43): n is a, c, g or t
  misc_feature (45)..(46): n is a, c, g or t
  misc_feature (48)..(49): n is a, c, g or t
attaggtcaccgtctcctcagagcccaaatcttgtnnknnknnknnknnktgcccaccgtgcccagcacctgaactcct

SEQ ID NO: 139 - DNA, 82 bp, Artificial Sequence
  Forward primer-6
  misc_feature (36)..(37): n is a, c, g or t
  misc_feature (39)..(40): n is a, c, g or t
  misc_feature (42)..(43): n is a, c, g or t
  misc_feature (45)..(46): n is a, c, g or t
  misc_feature (48)..(49): n is a, c, g or t
  misc_feature (51)..(52): n is a, c, g or t
attaggtcaccgtctcctcagagcccaaatcttgtnnknnknnknnknnknnktgcccaccgtgcccagcacctgaactcct

SEQ ID NO: 140 - DNA, 85 bp, Artificial Sequence
  Forward primer-7
  misc_feature (36)..(37): n is a, c, g or t
  misc_feature (39)..(40): n is a, c, g or t
  misc_feature (42)..(43): n is a, c, g or t
  misc_feature (45)..(46): n is a, c, g or t
  misc_feature (48)..(49): n is a, c, g or t
  misc_feature (51)..(52): n is a, c, g or t
  misc_feature (54)..(55): n is a, c, g or t
attaggtcaccgtctcctcagagcccaaatcttgtnnknnknnknnknnknnknnktgcccaccgtgcccagcacctgaactcct

SEQ ID NO: 141 - DNA, 88 bp, Artificial Sequence
  Forward primer-8
  misc_feature (36)..(37): n is a, c, g or t
  misc_feature (39)..(40): n is a, c, g or t
  misc_feature (42)..(43): n is a, c, g or t
  misc_feature (45)..(46): n is a, c, g or t
  misc_feature (48)..(49): n is a, c, g or t
  misc_feature (51)..(52): n is a, c, g or t
  misc_feature (54)..(55): n is a, c, g or t
  misc_feature (57)..(58): n is a, c, g or t
attaggtcaccgtctcctcagagcccaaatcttgtnnknnknnknnknnknnknnknnktgcccaccgtgcccagcacctgaactcct

SEQ ID NO: 142 - DNA, 91 bp, Artificial Sequence
  Forward primer-9
  misc_feature (36)..(37): n is a, c, g or t
  misc_feature (39)..(40): n is a, c, g or t
  misc_feature (42)..(43): n is a, c, g or t
  misc_feature (45)..(46): n is a, c, g or t
  misc_feature (48)..(49): n is a, c, g or t
  misc_feature (51)..(52): n is a, c, g or t
  misc_feature (54)..(55): n is a, c, g or t
  misc_feature (57)..(58): n is a, c, g or t
  misc_feature (60)..(61): n is a, c, g or t
attaggtcaccgtctcctcagagcccaaatcttgtnnknnknnknnknnknnknnknnknnktgcccaccgtgcccagcacctgaactcct

SEQ ID NO: 143 - DNA, 94 bp, Artificial Sequence
  Forward primer-10
  misc_feature (36)..(37): n is a, c, g or t
  misc_feature (39)..(40): n is a, c, g or t
  misc_feature (42)..(43): n is a, c, g or t
  misc_feature (45)..(46): n is a, c, g or t
  misc_feature (48)..(49): n is a, c, g or t
  misc_feature (51)..(52): n is a, c, g or t
  misc_feature (54)..(55): n is a, c, g or t
  misc_feature (57)..(58): n is a, c, g or t
  misc_feature (60)..(61): n is a, c, g or t
  misc_feature (63)..(64): n is a, c, g or t
attaggtcaccgtctcctcagagcccaaatcttgtnnknnknnknnknnknnknnknnknnknnktgcccaccgtgcccagcacctgaactcct

SEQ ID NO: 144 - DNA, 24 bp, Artificial Sequence
  Reverse primer
actcgactcgagtcccccgggatg

SEQ ID NO: 145 - protein, 15 aa, Artificial Sequence
  Human IgG1 hinge region var. (GS)2-C220
GSGSCDKTHTCPPCP

SEQ ID NO: 146 - protein, 16 aa, Artificial Sequence
  Human IgG1 hinge region var. (G4S)-C220
GGGGSCDKTHTCPPCP

SEQ ID NO: 147 - protein, 21 aa, Mus musculus
  Mouse IgG2c hinge region
EPRVPITQNPCPPLKECPPCA

SEQ ID NO: 148 - protein, 360 aa, Artificial Sequence
  PR006468 chain
EVQLVETGGGLIQPGGSLRLSCAASGFTVSDSYMTWVRQAPGKGLEWVSVIFSGGRTYYSDSVKGRFTISRDNAKNTLYLQMNSLRAEDTALYYCARRNYDDTRGTDVFDIWGQGTMVTVSSEPRVPITQNPCPPLKECPPCAAPELLGGPSVFLFPPKPKDTLMISRTPEVTCVVVDVSHEDPEVKFNWYVDGVEVHNAKTKPREEQYNSTYRVVSVLTVLHQDWLNGKEYKCKVSNKALPAPIEKTISKAKGQPREPQVYTLPPSREEMTKNQVSLTCLVKGFYPSDIAVEWESNGQPENNYKTTPPVLDSDGSFFLYSKLTVDKSRWQQGNVFSCSVMHEALHNHYTQKSLSLSPGK

SEQ ID NO: 149 - protein, 356 aa, Artificial Sequence
  PR006345 chain
EEELQIIQPDKSVLVAAGETATLRCTITSLFPVGPIQWFRGAGPGRVLIYNQRQGPFPRVTTVSDTTKRNNMDFSIRIGNITPADAGTYYCIKFRKGSPDDVEFKSGAGTELSVRAKPSGGGASEPKSCDKTHTCPPCPAPELLGGPSVFLFPPKPKDTLMISRTPEVTCVVVDVSHEDPEVKFNWYVDGVEVHNAKTKPREEQYNSTYRVVSVLTVLHQDWLNGKEYKCKVSNKALPAPIEKTISKAKGQPREPQVYTLPPSREEMTKNQVSLTCLVKGFYPSDIAVEWESNGQPENNYKTTPPVLDSDGSFFLYSKLTVDKSRWQQGNVFSCSVMHEALHNHYTQKSLSLSPGK